European Patent Application EP 4 112 639 A1, published January 4, 2023. Title: CAR T/NK-CELLS FOR USE IN THE TREATMENT OF FUNGAL INFECTIONS. Applicant: Universitat de Barcelona Hospital Clínic de Barcelona Institut d’Investigacions Biomèdiques August Pi i Sunyer (IDIBAPS). The sequence listing filed with the application follows.

SEQUENCE LISTING (16 sequences)

SEQ ID NO: 1 - protein, 345 aa, Artificial sequence
  Artificial sequence
  MISC_FEATURE (200)..(200): P or L
RLSWYDPDFQARLTRSNSKCQGQLEVYLKDGWHMVCSQSWGRSSKQWEDPSQASKVCQRLNCGVPLSLGPFLVTYTPQSSIICYGQLGSFSNCSHSRNDMCHSLGLTCLEPQKTTPPTTRPPPTTTPEPTAPPRLQLVAQSGGQHCAGVVEFYSGSLGGTISYEAQDKTQDLENFLCNNLQCGSFLKHLPETEAGRAQDPGEPREHQPLPIQWKIQNSSCTSLEHCFRKIKPQKSGRVLALLCSGFQPKVQSRLVGGSSICEGTVEVRQGAQWAALCDSSSARSSLRWEEVCREQQCGSVNSYRVLDAGDPTSRGLFCPHQKLSQCHELWERNSYCKKVFVTCQD

SEQ ID NO: 2 - protein, 372 aa, Artificial sequence
  Artificial sequence
  MISC_FEATURE (224)..(224): P or L
MPMGSLQPLATLYLLGMLVASCLGRLSWYDPDFQARLTRSNSKCQGQLEVYLKDGWHMVCSQSWGRSSKQWEDPSQASKVCQRLNCGVPLSLGPFLVTYTPQSSIICYGQLGSFSNCSHSRNDMCHSLGLTCLEPQKTTPPTTRPPPTTTPEPTAPPRLQLVAQSGGQHCAGVVEFYSGSLGGTISYEAQDKTQDLENFLCNNLQCGSFLKHLPETEAGRAQDPGEPREHQPLPIQWKIQNSSCTSLEHCFRKIKPQKSGRVLALLCSGFQPKVQSRLVGGSSICEGTVEVRQGAQWAALCDSSSARSSLRWEEVCREQQCGSVNSYRVLDAGDPTSRGLFCPHQKLSQCHELWERNSYCKKVFVTCQDPNP

SEQ ID NO: 3 - protein, 21 aa, Artificial sequence
  Artificial sequence
MALPVTGLLLSLGLLLHAARP

SEQ ID NO: 4 - protein, 46 aa, Artificial sequence
  Artificial sequence
TTTPAPRPPTPAPTIASQPLSLRPEACRPAAGGAVHTRGLDFACDI

SEQ ID NO: 5 - protein, 23 aa, Artificial sequence
  Artificial sequence
YIWAPLAGTCGVLLLSLVITLYC

SEQ ID NO: 6 - protein, 23 aa, Artificial sequence
  Artificial sequence
PFFFCCFIAVAMGIRFIIMVAIW

SEQ ID NO: 7 - protein, 42 aa, Artificial sequence
  Artificial sequence
KRGRKKLLYIFKQPFMRPVQTTQEEDGCSCRFPEEEEGGCEL

SEQ ID NO: 8 - protein, 41 aa, Artificial sequence
  Artificial sequence
RSKRSRLLHSDYMNMTPRRPGPTRKHYQPYAPPRDFAAYRS

SEQ ID NO: 9 - protein, 120 aa, Artificial sequence
  Artificial sequence
WRRKRKEKQSETSPKEFLTIYEDVKDLKTRRNHEQEQTFPGGGSTIYSMIQSQSSAPTSQEPAYTLYSLIQPSRKSGSRKRNHSPSFNSTIYEVIGKSQPKAQNPARLSRKELENFDVYS

SEQ ID NO: 10 - protein, 113 aa, Artificial sequence
  Artificial sequence
RVKFSRSADAPAYQQGQNQLYNELNLGRREEYDVLDKRRGRDPEMGGKPQRRKNPQEGLYNELQKDKMAEAYSEIGMKGERRRGKGHDGLYQGLSTATKDTYDALHMQALPPR

SEQ ID NO: 11 - protein, 590 aa, Artificial sequence
  Artificial sequence
  MISC_FEATURE (221)..(221): P or L
MALPVTGLLLSLGLLLHAARPRLSWYDPDFQARLTRSNSKCQGQLEVYLKDGWHMVCSQSWGRSSKQWEDPSQASKVCQRLNCGVPLSLGPFLVTYTPQSSIICYGQLGSFSNCSHSRNDMCHSLGLTCLEPQKTTPPTTRPPPTTTPEPTAPPRLQLVAQSGGQHCAGVVEFYSGSLGGTISYEAQDKTQDLENFLCNNLQCGSFLKHLPETEAGRAQDPGEPREHQPLPIQWKIQNSSCTSLEHCFRKIKPQKSGRVLALLCSGFQPKVQSRLVGGSSICEGTVEVRQGAQWAALCDSSSARSSLRWEEVCREQQCGSVNSYRVLDAGDPTSRGLFCPHQKLSQCHELWERNSYCKKVFVTCQDTTTPAPRPPTPAPTIASQPLSLRPEACRPAAGGAVHTRGLDFACDIYIWAPLAGTCGVLLLSLVITLYCKRGRKKLLYIFKQPFMRPVQTTQEEDGCSCRFPEEEEGGCELRVKFSRSADAPAYQQGQNQLYNELNLGRREEYDVLDKRRGRDPEMGGKPQRRKNPQEGLYNELQKDKMAEAYSEIGMKGERRRGKGHDGLYQGLSTATKDTYDALHMQALPPR

SEQ ID NO: 12 - protein, 631 aa, Artificial sequence
  Artificial sequence
  MISC_FEATURE (221)..(221): P or L
MALPVTGLLLSLGLLLHAARPRLSWYDPDFQARLTRSNSKCQGQLEVYLKDGWHMVCSQSWGRSSKQWEDPSQASKVCQRLNCGVPLSLGPFLVTYTPQSSIICYGQLGSFSNCSHSRNDMCHSLGLTCLEPQKTTPPTTRPPPTTTPEPTAPPRLQLVAQSGGQHCAGVVEFYSGSLGGTISYEAQDKTQDLENFLCNNLQCGSFLKHLPETEAGRAQDPGEPREHQPLPIQWKIQNSSCTSLEHCFRKIKPQKSGRVLALLCSGFQPKVQSRLVGGSSICEGTVEVRQGAQWAALCDSSSARSSLRWEEVCREQQCGSVNSYRVLDAGDPTSRGLFCPHQKLSQCHELWERNSYCKKVFVTCQDTTTPAPRPPTPAPTIASQPLSLRPEACRPAAGGAVHTRGLDFACDIYIWAPLAGTCGVLLLSLVITLYCRSKRSRLLHSDYMNMTPRRPGPTRKHYQPYAPPRDFAAYRSKRGRKKLLYIFKQPFMRPVQTTQEEDGCSCRFPEEEEGGCELRVKFSRSADAPAYQQGQNQLYNELNLGRREEYDVLDKRRGRDPEMGGKPQRRKNPQEGLYNELQKDKMAEAYSEIGMKGERRRGKGHDGLYQGLSTATKDTYDALHMQALPPR

SEQ ID NO: 13 - protein, 668 aa, Artificial sequence
  Artificial sequence
  MISC_FEATURE (221)..(221): P or L
MALPVTGLLLSLGLLLHAARPRLSWYDPDFQARLTRSNSKCQGQLEVYLKDGWHMVCSQSWGRSSKQWEDPSQASKVCQRLNCGVPLSLGPFLVTYTPQSSIICYGQLGSFSNCSHSRNDMCHSLGLTCLEPQKTTPPTTRPPPTTTPEPTAPPRLQLVAQSGGQHCAGVVEFYSGSLGGTISYEAQDKTQDLENFLCNNLQCGSFLKHLPETEAGRAQDPGEPREHQPLPIQWKIQNSSCTSLEHCFRKIKPQKSGRVLALLCSGFQPKVQSRLVGGSSICEGTVEVRQGAQWAALCDSSSARSSLRWEEVCREQQCGSVNSYRVLDAGDPTSRGLFCPHQKLSQCHELWERNSYCKKVFVTCQDTTTPAPRPPTPAPTIASQPLSLRPEACRPAAGGAVHTRGLDFACDIPFFFCCFIAVAMGIRFIIMVAIWWRRKRKEKQSETSPKEFLTIYEDVKDLKTRRNHEQEQTFPGGGSTIYSMIQSQSSAPTSQEPAYTLYSLIQPSRKSGSRKRNHSPSFNSTIYEVIGKSQPKAQNPARLSRKELENFDVYSRVKFSRSADAPAYQQGQNQLYNELNLGRREEYDVLDKRRGRDPEMGGKPQRRKNPQEGLYNELQKDKMAEAYSEIGMKGERRRGKGHDGLYQGLSTATKDTYDALHMQALPPR

SEQ ID NO: 14 - DNA, 1773 bp, Artificial sequence
  Artificial sequence
atggccttaccagtgaccggcttgctcctgtcgctgggcttgctgctccacgccgccaggccgagactgagttggtacgatcccgacttccaggcacgactgacacggagtaatagtaaatgccaggggcagctggaggtgtatctgaaagacggatggcacatggtgtgcagtcagtcatggggccggagctccaagcagtgggaggatccttcccaggcctctaaagtgtgccagagactgaactgtggagtccctctgtccctgggcccattcctggtcacatacactccacagtctagtatcatttgctatggccagctggggagcttttccaactgttctcacagtaggaatgacatgtgccattctctggggctgacttgtctggagccccagaagaccacaccacctactacccgaccaccacctacaactacccctgaaccaaccgctccaccacgactgcagctggtggcacagagcggaggacagcactgtgccggagtggtcgagttctactcaggcagcctgggaggcaccatcagctatgaggcccaggacaagacacaggatctggaaaacttcctgtgcaacaatctgcagtgtggcagctttctgaaacacctgcctgagacagaagcagggagggcacaggacccaggagagccacgagaacatcagcccctgcctatccagtggaaaattcagaattcaagctgcacttccctggagcattgtttccgaaagatcaaaccacagaagtctggacgggtgctggccctgctgtgcagcggatttcagcccaaagtgcagtccaggctggtcgggggatcctctatttgcgaggggacagtggaagtccgccagggagctcagtgggccgccctgtgcgatagttcaagcgcacggtcctctctgagatgggaggaagtgtgccgggaacagcagtgtggcagtgtgaattcatacagagtcctggacgctggcgatcccacctctagggggctgttttgtcctcatcagaagctgagtcagtgtcacgaactgtgggaacggaactcatactgtaaaaaggtgtttgtcacttgccaggatacaactacgccggcgccgagaccacctacacctgcaccaactattgcctctcagccactgagtctgcgccccgaggcatgtcgacctgccgctggcggggctgtgcacaccaggggcctagacttcgcctgcgatatctatatttgggctccactggcaggaacctgtggcgtgctgctgctgtctctggtcatcacactgtactgcaaaagaggcaggaagaaactgctgtatattttcaagcagccctttatgagacctgtgcagacaactcaggaggaagacgggtgcagctgtaggttccctgaggaagaggaaggaggctgtgagctgcgcgtgaaattttctcggagtgcagatgccccagcttaccagcagggccagaaccagctgtataacgagctgaatctggggcggagagaggaatacgacgtgctggataagaggcgcgggcgagatccagaaatgggaggaaaaccccagcgacggaagaaccctcaggagggactgtacaatgaactgcagaaggacaaaatggcagaggcctattccgaaatcgggatgaaaggagaaagaaggcgcggcaaggggcatgatggcctgtatcagggactgtcaaccgcaacaaaagatacttatgatgctctgcacatgcaggctctgcccccgcggtaa

SEQ ID NO: 15 - DNA, 1932 bp, Artificial sequence
  Artificial sequence
atggccctgcccgtgaccggactgctgctgagcctgggcctgctgctgcacgccgctaggccaaggctgagctggtacgatcctgactttcaggccaggctgaccaggtccaattccaagtgtcagggccagctggaggtgtacctgaaggacggctggcacatggagacagtgtgttcccagagctggggcagatccagcaagcagtgggaggaccctagccaggcctccaaggtgtgccagaggctgaattgcggcgtgcccctgagcctgggacctttcctggtgacctacaccccccagtccagcatcatctgttacggccagctgggctccttttccaactgcagccactccaggaatgatatggagacctgccacagcctgggcctcacctgtctggagccccagaagacaacaccccctaccacaagacctccccctaccaccacccctgagcccaccgctccccctagactgcagctggtggcccagagcggcggccaacactgcgctggagtggtggagttctacagcggcagcctgggcggcacaatcagctacgaggcccaggataagacccaggatctggagaactttctgtgcaacaatctgcagtgtggcagctttctgaagcacctgcctgagacagaggccggcagggcccaggatcctggcgaaccaagagagcaccagcccctgcctatccagtggaagatccagaatagctcctgcacctccctggagcactgttttagaaagatcaagccccagaagagcggcagagtgctggccctgctgtgtagcggcttccagcccaaggtgcagagcaggctggtgggcggctcctccatctgcgagggcacagtggaggtgagacagggcgcccagtgggccgctctgtgtgatagcagcagcgccagatccagcctgaggtgggaggaggtgtgcagggagcagcagtgtggctccgtgaactcctacagggtgctggatgccggcgatcctacatccaggggcctgttttgtccccaccagaagctgagccagtgccacgagctgtgggagaggaattcctactgcaagaaggtgttcgtgacatgtcaggacacaaccacccctgcccccagacctcctacacccgcccctaccatcgcctcccagcccctgagcctcaggcccgaagcctgtagacctgccgccggcggagccgttcacaccagaggactggatttcgcctgcgatatctacatctgggcccccctggccggcacctgtggagttctgctgctgtccctggtcattaccctgtactgtagaagcaagagaagcaggctgctgcactccgattacatgaatatgacccctagaagacctggccctaccaggaagcactaccagccttacgcccctcccagggactttgccgcctacagatccaagagaggcagaaagaagctgctgtacatctttaagcagccttttatggagacaagacctgtgcagaccacccaggaggaggacggctgctcctgcagatttcctgaggaggaggagggcggctgtgagctgagggtgaagtttagcaggtccgccgatgcccctgcctaccagcagggccagaaccagctgtacaatgagctgaacctgggcagaagggaggagtacgacgtgctggataagagaaggggcagggatcctgagatggagaccggcggcaagccccagagaaggaagaatccccaggagggcctgtacaatgaactgcagaaggacaagatggagacagccgaggcctacagcgagatcggcatggagaccaagggcgagagaagaaggggcaagggccacgacggcctgtaccagggcctgagcacagccaccaaggatacatacgacgccctgcacatgcaggccctgccccctagatga

SEQ ID NO: 16 - DNA, 2019 bp, Artificial sequence
  Artificial sequence
atggccctgcccgtgacaggcctgctgctgagcctgggcctgctgctccacgccgctagacccagactgagctggtacgatcccgactttcaggccaggctgacaagaagcaacagcaagtgtcagggccagctggaggtgtacctgaaggatggctggcacatggagacagtgtgcagccagtcctggggcaggtcctccaagcagtgggaggatccttcccaggccagcaaggtgtgtcagagactgaattgcggcgtgcccctgagcctgggaccctttctggtgacatacacccctcagagcagcatcatctgctacggccagctgggctcctttagcaattgctcccactccaggaatgatatggagacatgccacagcctgggcctcacctgcctggagccccagaagaccacaccccccaccaccaggccccctcctaccacaacccctgagcccaccgcccctcccagactgcagctggtggcccagagcggcggccaacactgcgctggagtggtggagttttacagcggcagcctgggcggcacaatcagctacgaggcccaggacaagacccaggacctggagaattttctgtgtaataatctgcagtgtggctccttcctgaagcacctgcccgagacagaggccggcagagcccaggaccccggagaacctagggagcaccagcccctgcccatccagtggaagatccagaacagctcctgtacatccctggagcactgcttcaggaagatcaagccccagaagtccggcagagtgctggccctgctgtgttccggcttccagcccaaggtgcagtccaggctggtgggcggctccagcatctgcgagggcacagtggaggtgagacagggcgcccagtgggccgctctgtgtgatagctccagcgccagaagcagcctgaggtgggaggaggtgtgcagagagcagcagtgtggcagcgtgaattcctacagagtgctggacgccggcgatcctacaagcaggggcctgttttgtccccaccagaagctgtcccagtgccacgagctgtgggagagaaatagctactgtaagaaggtgtttgtgacctgtcaggacacaaccacccccgcccccaggccaccaacccctgctcctaccatcgccagccagcctctgtccctgagacccgaggcctgtaggcctgccgccggaggagctgtgcacaccagaggcctggatttcgcctgcgatatccccttcttcttttgctgcttcatcgccgtggccatgggcatcagattcatcatcatggtggccatctggtggaggaggaagagaaaggagaagcagtccgagacaagccccaaggagttcctgacaatctacgaggatgtgaaggatctgaagaccaggagaaatcacgagcaggagcagacatttcctggcggcggcagcaccatctactccatgatccagtcccagtcctccgcccctacatcccaggagcccgcctacacactgtactccctgatccagcctagcagaaagagcggctccagaaagagaaaccacagcccttccttcaactccacaatctacgaagtgatcggcaagagccagcccaaggcccagaatcccgccagactgagcaggaaggagctggagaatttcgatgtgtactccagagtgaagttttccaggagcgccgacgcccccgcctaccaacagggacagaatcagctgtacaatgagctgaacctgggcaggagggaggagtacgacgtgctggacaagagaagaggcagggaccctgagatgggcggcaagcctcagagaaggaagaatcctcaggagggcctgtacaacgagctgcagaaggacaagatggccgaggcctactccgagatcggcatgaagggcgagaggagaaggggcaagggccacgacggcctgtaccagggcctgtccaccgccaccaaggatacatacgatgccctgcacatgcaggccctgccccccagatga